European Patent Specification EP 3 839 070 B1, published July 22, 2026. Title: DNA Methylation Related Markers For Diagnosis Of Tumors And Application Thereof. Applicant: SHANGHAI PUBLIC HEALTH CLINICAL CENTER. The sequence listing filed with the application follows.

SEQUENCE LISTING (21 sequences)

SEQ ID NO: 1 - DNA, 699 bp, Homo sapiens
cgcccagtaagttacggaaaaggcggagacagaggtttcgttcccgcccctccaattcagtctccaaaaaggtccgcataattgatatataaggggcttcagtgtgtagcaaagttgcaaaagttaagagttgttgtttgtcttcgatcatgtctggtagaggcaaaggtggtaaaggtttaggaaagggaggcgccaagcgccatcgcaaagtgctgcgtgacaacatacagggcatcacgaagcccgccatccgtcgcttggcccgacgcggcggcgtgaaacgcatttcgggcctcatttatgaggagacccgcggtgttcttaaggtgttcctggagaatgtgatacgggacgccgtaacctacacggagcacgccaagcgtaagacagtcactgcaatggatgttgtctacgcgctcaagcgccagggacgcactctgtacggctttggtggctgagcctcaccccggctttttatttaacagctcacccataaaaggcccttttcagggccacctccttcgtcacacgaagggctgtaactgatgacgacttgggtttcgttttgtaaatttgggattctaactgagttaaaccgagccgtttttagcgatcttcctaagatggcggatgtgctaaggagaaagggaaggcgaaacattagaaacttgttcaggtatttcgatcgcaaacatt

SEQ ID NO: 2 - DNA, 699 bp, Artificial Sequence
  misc_feature (1)..(699): bisulfite treated sequence
  misc_feature (1)..(699): y is c or t
ygtttagtaagttayggaaaaggyggagatagaggtttygttttygtttttttaatttagtttttaaaaaggttygtataattgatatataaggggttttagtgtgtagtaaagttgtaaaagttaagagttgttgtttgttttygattatgtttggtagaggtaaaggtggtaaaggtttaggaaagggaggygttaagygttatygtaaagtgttgygtgataatatatagggtattaygaagttygttattygtygtttggttygaygyggyggygtgaaaygtatttygggttttatttatgaggagattygyggtgtttttaaggtgtttttggagaatgtgataygggaygtygtaatttatayggagtaygttaagygtaagatagttattgtaatggatgttgtttaygygtttaagygttagggaygtattttgtayggttttggtggttgagttttatttyggttttttatttaatagtttatttataaaaggttttttttagggttatttttttygttataygaagggttgtaattgatgaygatttgggtttygttttgtaaatttgggattttaattgagttaaatygagtygtttttagygatttttttaagatggyggatgtgttaaggagaaagggaaggygaaatattagaaatttgtttaggtatttygatygtaaatatt

SEQ ID NO: 3 - DNA, 624 bp, Homo sapiens
agctgtttgttaaataggctttcattttaattttttaaaaaatattttcactagttagacggaatatttatttctgatcctcgttgtagggctaaactaggtgtgacttgcttttccattaaggactgtagccattttggctaagaaagtctttcctgtcttagctctcttcaagagatgctatttacttttttgttgttgttttctccggagctttattgcctaccctttattttcacgatgtgtttgtgcattctgtaaaaagtgggaaacactgttctccggattgtgtgggtgatcgccggtcgcctagcttgccgttcttcaggtatctcctgctgctccagaatctacatctgaatgtcaaggcatagcttttccaggagcttttaaaccgacctttcaattcgaagacgtaactgcgccaggagctttgtctccctggcatataaaagcatagaagagagcaacttctggtttttaaaataagtaaactaatctgaattgtttgcaatggtaggaacttgttatataaaatgttaattaggtggcccgtgctcgaaaactgctctcaggatatgaccaatgggagagtagacctaagctccttcatttgcatgcaga

SEQ ID NO: 4 - DNA, 624 bp, Artificial Sequence
  misc_feature (1)..(624): bisulfite treated sequence
  misc_feature (1)..(624): y is c or t
agttgtttgttaaataggtttttattttaattttttaaaaaatatttttattagttagayggaatatttatttttgattttygttgtagggttaaattaggtgtgatttgtttttttattaaggattgtagttattttggttaagaaagttttttttgttttagttttttttaagagatgttatttatttttttgttgttgtttttttyggagttttattgtttattttttatttttaygatgtgtttgtgtattttgtaaaaagtgggaaatattgtttttyggattgtgtgggtgatygtyggtygtttagtttgtygttttttaggtattttttgttgttttagaatttatatttgaatgttaaggtatagtttttttaggagtttttaaatygattttttaattygaagaygtaattgygttaggagttttgtttttttggtatataaaagtatagaagagagtaatttttggtttttaaaataagtaaattaatttgaattgtttgtaatggtaggaatttgttatataaaatgttaattaggtggttygtgttygaaaattgtttttaggatatgattaatgggagagtagatttaagtttttttatttgtatgtaga

SEQ ID NO: 5 - DNA, 669 bp, Homo sapiens
tggggcaactcatccaataagattgtctagtaatgaaccaatcagtctggtcactcttcagccaatgattttatcgcgcgggacttttgaaatattacaggaccaatcagaatgtttctcactatatttaaaggccacttgctctcagttcactacacttttgtgtgtgctctcattgcaaatggctcgtacgaagcaaacagctcgcaagtctaccggcggcaaagctccgcgcaagcagcttgctactaaagcagcccgtaagagcgctccggccaccggtggcgtgaagaaacctcatcgctaccgcccgggcaccgtggccttgcgcgaaatccgtcgctaccagaagtccaccgagctgctgatccggaagctgccgttccagcgcctggtgcgagaaatcgcccaggacttcaaaaccgacctgcgtttccagagctctgcggtgatggcgctgcaggaggcttgtgaggcctacctggtgggactcttcgaagacaccaatctgtgcgctattcacgctaaacgcgtcaccatcatgcccaaagatatccagctggcacgtcgcatccgtggggaaagggcataagtctgcccgtttcttcctcattgaaaaggctcttttcagagccactcacaatttcacttaaaaacagttgtaaccca

SEQ ID NO: 6 - DNA, 669 bp, Artificial Sequence
  misc_feature (1)..(669): bisulfite treated sequence
  misc_feature (1)..(669): y is c or t
tggggtaatttatttaataagattgtttagtaatgaattaattagtttggttattttttagttaatgattttatygygygggatttttgaaatattataggattaattagaatgttttttattatatttaaaggttatttgtttttagtttattatatttttgtgtgtgtttttattgtaaatggttygtaygaagtaaatagttygtaagtttatyggyggtaaagtttygygtaagtagtttgttattaaagtagttygtaagagygtttyggttatyggtggygtgaagaaattttatygttatygttygggtatygtggttttgygygaaattygtygttattagaagtttatygagttgttgattyggaagttgtygttttagygtttggtgygagaaatygtttaggattttaaaatygatttgygtttttagagttttgyggtgatggygttgtaggaggtttgtgaggtttatttggtgggatttttygaagatattaatttgtgygttatttaygttaaaygygttattattatgtttaaagatatttagttggtaygtygtattygtggggaaagggtataagtttgttygttttttttttattgaaaaggttttttttagagttatttataattttatttaaaaatagttgtaattta

SEQ ID NO: 7 - DNA, 374 bp, Homo sapiens
tacccataaaagaaagctgccatcacaggcagcagacctttgttctctgaccacttgataatgtcaggacgcggcaaaggaggtaagggcctggggaaagggggtgccaagcgccaccgcaaggtgctgcgcgacaacatccagggtatcaccaagccagccattcggcgccttgctcgccgcggcggcgtgaagcgcatttctggcctcatctatgaggagacccgcggagtgttgaaggtgttcctggagaacgtgatccgggacgccgtgacctacacggagcacgccaagcgcaagacggtcaccgccatggacgtggtctacgcgctcaagcgccagggccgcaccctctatggcttcggcggctaaat

SEQ ID NO: 8 - DNA, 374 bp, Artificial Sequence
  misc_feature (1)..(448): bisulfite treated sequence
  misc_feature (1)..(448): y is c or t
tatttataaaagaaagttgttattataggtagtagatttttgttttttgattatttgataatgttaggaygyggtaaaggaggtaagggtttggggaaagggggtgttaagygttatygtaaggtgttgygygataatatttagggtattattaagttagttattyggygttttgttygtygyggyggygtgaagygtatttttggttttatttatgaggagattygyggagtgttgaaggtgtttttggagaaygtgattygggaygtygtgatttatayggagtaygttaagygtaagayggttatygttatggaygtggtttaygygtttaagygttagggtygtattttttatggtttyggyggttaaat

SEQ ID NO: 9 - DNA, 27 bp, Primer
gtagaggtaaaggtggtaaaggtttag

SEQ ID NO: 10 - DNA, 50 bp, Primer
aaccttcaacaccccaaccatataaaaacaccrcraatctcctcataaat

SEQ ID NO: 11 - DNA, 26 bp, Primer
tgttgygtgataatatatagggtatt

SEQ ID NO: 12 - DNA, 24 bp, Primer
aaccttcaacaccccaaccatata

SEQ ID NO: 13 - DNA, 28 bp, Primer
gatgtgtttgtgtattttgtaaaaagtg

SEQ ID NO: 14 - DNA, 51 bp, Primer
aaccttcaacaccccaaccatatatataccttaacattcaaatataaattc

SEQ ID NO: 15 - DNA, 20 bp, Primer
ttttyggattgtgtgggtga

SEQ ID NO: 16 - DNA, 30 bp, Primer
tttgtttttagtttattatatttttgtgtg

SEQ ID NO: 17 - DNA, 50 bp, Primer
aaccttcaacaccccaaccatataaactactttaataacaaactacttac

SEQ ID NO: 18 - DNA, 23 bp, Primer
gtgtgtgtttttattgtaaatgg

SEQ ID NO: 19 - DNA, 28 bp, Primer
gggtgttaagygttatygtaaggtgttg

SEQ ID NO: 20 - DNA, 50 bp, Primer
aaccttcaacaccccaaccatatactcctcataaataaaaccaaaaatac

SEQ ID NO: 21 - DNA, 24 bp, Primer
tttagggtattattaagttagtta